European Patent Application EP 4 230 736 A1, published August 23, 2023. Title: METHOD OF DETECTING GENE POLYMORPHISM. Applicant: SHIMADZU CORPORATION NATIONAL CEREBRAL AND CARDIOVASCULAR CENTER. The sequence listing filed with the application follows.

SEQUENCE LISTING (14 sequences)

SEQ ID NO: 1 - DNA, 17 bp, Artificial Sequence
  Synthesized oligonucleotide to act as a PCR forward primer to amplify ApoE gene fragment containing the codon corresponding to the 112th amino acid residue.
caaggagctgcaggcgg

SEQ ID NO: 2 - DNA, 18 bp, Artificial Sequence
  Synthesized oligonucleotide to act as a PCR reverse primer to amplify ApoE gene fragment containing the codon corresponding to the 112th amino acid residue.
cagctcctcggtgctctg

SEQ ID NO: 3 - DNA, 15 bp, Artificial Sequence
  Synthesized oligonucleotide to act as a PCR forward primer to amplify ApoE gene fragment containing the codon corresponding to the 112th amino acid residue.
ggcgcaggcccggct

SEQ ID NO: 4 - DNA, 14 bp, Artificial Sequence
  Synthesized oligonucleotide to act as a PCR reverse primer to amplify ApoE gene fragment containing the codon corresponding to the 112th amino acid residue.
cggcgccctcgcgg

SEQ ID NO: 5 - DNA, 17 bp, Artificial Sequence
  Synthesized oligonucleotide to act as a PCR forward primer to amplify ApoE gene fragment containing the codon corresponding to the 158th amino acid residue.
cgcaagctgcgtaagcg

SEQ ID NO: 6 - DNA, 16 bp, Artificial Sequence
  Synthesized oligonucleotide to act as a PCR reverse primer to amplify ApoE gene fragment containing the codon corresponding to the 158th amino acid residue.
cgcggatggcgctgag

SEQ ID NO: 7 - DNA, 17 bp, Artificial Sequence
  Synthesized oligonucleotide to act as a PCR forward primer to amplify ApoE gene fragment containing the codon corresponding to the 158th amino acid residue.
cgtaagcggctcctccg

SEQ ID NO: 8 - DNA, 14 bp, Artificial Sequence
  Synthesized oligonucleotide to act as a PCR reverse primer to amplify ApoE gene fragment containing the codon corresponding to the 158th amino acid residue.
cggcgccctcgcgg

SEQ ID NO: 9 - DNA, 15 bp, Artificial Sequence
  Synthesized oligonucleotide to act as a probe to detect amplified ApoE gene fragment containing the wild-type gene polymorphism corresponding to the 112th amino acid residue.
ggacgtgtgcggccg

SEQ ID NO: 10 - DNA, 15 bp, Artificial Sequence
  Synthesized oligonucleotide to act as a probe to detect amplified ApoE gene fragment containing the mutant gene polymorphism corresponding to the 112th amino acid residue.
ggacgtgcgcggccg

SEQ ID NO: 11 - DNA, 17 bp, Artificial Sequence
  Synthesized oligonucleotide to act as a probe to detect amplified ApoE gene fragment containing the wild-type gene polymorphism corresponding to the 158th amino acid residue.
ctgcagaagcgcctggc

SEQ ID NO: 12 - DNA, 17 bp, Artificial Sequence
  Synthesized oligonucleotide to act as a probe to detect amplified ApoE gene fragment containing the mutant gene polymorphism corresponding to the 158th amino acid residue.
ctgcagaagtgcctggc

SEQ ID NO: 13 - DNA, 244 bp, Homo sapiens
  misc_feature: ApoE gene sequence of the region containing the gene polymorphism corresponding to the 112th amino acid residue.
  variation (122)..(124): The wild-type codon corresponding to the 112th amino acid residue.
gaaggcctacaaatcggaactggaggaacaactgaccccggtggcggaggagacgcgggcacggctgtccaaggagctgcaggcggcgcaggcccggctgggcgcggacatggaggacgtgtgcggccgcctggtgcagtaccgcggcgaggtgcaggccatgctcggccagagcaccgaggagctgcgggtgcgcctcgcctcccacctgcgcaagctgcgtaagcggctcctccgcgatgcc

SEQ ID NO: 14 - DNA, 208 bp, Homo sapiens
  misc_feature: ApoE gene sequence of the region containing the gene polymorphism corresponding to the 158th amino acid residue
  variation (135)..(137): The wild-type codon corresponding to the 158th amino acid residue.
gccgcctggtgcagtaccgcggcgaggtgcaggccatgctcggccagagcaccgaggagctgcgggtgcgcctcgcctcccacctgcgcaagctgcgtaagcggctcctccgcgatgccgatgacctgcagaagcgcctggcagtgtaccaggccggggcccgcgagggcgccgagcgcggcctcagcgccatccgcgagcgcctggg